European Patent Application EP 4 512 827 A2, published February 26, 2025. Title: COMPOSITIONS AND METHODS FOR TREATING AUTOIMMUNE DISEASES AND CANCERS. Applicant: YALE UNIVERSITY. Application JP 2023-81549, filed November 9, 2016. The sequence listing filed with the application follows.

SEQUENCE LISTING (6 sequences)

SEQ ID NO: 1 - DNA, 1523 bp, Homo sapiens
  misc_feature 1..1523: note = Homo sapiens sialic acid binding Ig-like lectin 15 (SIGLEC15), mRNA
  source 1..1523: mol_type = genomic DNA
tccggctcccgcagagcccacagggacctgcagatctgagtgccctgcccacccccgcccgccttccttcccccaccacgcctgggagggccctcactggggaggtggccgagagcgggtctggcctggggtgttcagatgctcacagcatggaaaagtccatctggctgctggcctgcttggcgtgggttctcccgacaggctcatttgtgagaactaaaatagatactacggagaacttgctcaacacagaggtgcacagctcgccagcgcagcgctggtccatgcaggtgccacccgaggtgagcgcggaggcaggcgacgcggcagtgctgccctgcaccttcacgcacccgcaccgccactacgacgggccgctgacggccatctggcgcgcgggcgagccctatgcgggcccgcaggtgttccgctgcgctgcggcgcggggcagcgagctctgccagacggcgctgagcctgcacggccgcttccggctgctgggcaacccgcgccgcaacgacctctcgctgcgcgtcgagcgcctcgccctggctgacgaccgccgctacttctgccgcgtcgagttcgccggcgacgtccatgaccgctacgagagccgccacggcgtccggctgcacgtgacagccgcgccgcggatcgtcaacatctcggtgctgcccagtccggctcacgccttccgcgcgctctgcactgccgaaggggagccgccgcccgccctcgcctggtccggcccggccctgggcaacagcttggcagccgtgcggagcccgcgtgagggtcacggccacctagtgaccgccgaactgcccgcactgacccatgacggccgctacacgtgtacggccgccaacagcctgggccgctccgaggccagcgtctacctgttccgcttccatggcgccagcggggcctcgacggtcgccctcctgctcggcgctctcggcttcaaggcgctgctgctgctcggggtcctggccgcccgcgctgcccgccgccgcccagagcatctggacaccccggacaccccaccacggtcccaggcccaggagtccaattatgaaaatttgagccagatgaacccccggagcccaccagccaccatgtgctcaccgtgaggagtccctcagccaccaacatccatttcagcactgtaaagaacaaaggccagtgcgaggcttggctggcacagccagtcctggttctcgggcaccttggcagcccccagctgggtggctcctcccctgctcaaggtcaagaccctgctcaaggaggctcatctggcctcctatgtggacaaccatttcggagctccctgatatttttgccagcatttcgtaaatgtgcatacgtctgtgtgtgtgtgtgtgtgtgagagagagagagagagagtacacgcattagcttgagcgtgaaacttccagaaatgttcccttgccctttcttacctagaacacctgctatagtaaagcagacaggaaactgttaaaaaaaaaaaaaaaaaa

SEQ ID NO: 2 - protein, 328 aa, Homo sapiens
  REGION 1..328: note = misc_feature - Sialic acid-binding Ig-like lectin 15 precursor
MEKSIWLLACLAWVLPTGSFVRTKIDTTENLLNTEVHSSPAQRWSMQVPPEVSAEAGDAAVLPCTFTHPHRHYDGPLTAIWRAGEPYAGPQVFRCAAARGSELCQTALSLHGRFRLLGNPRRNDLSLRVERLALADDRRYFCRVEFAGDVHDRYESRHGVRLHVTAAPRIVNISVLPSPAHAFRALCTAEGEPPPALAWSGPALGNSLAAVRSPREGHGHLVTAELPALTHDGRYTCTAANSLGRSEASVYLFRFHGASGASTVALLLGALGFKALLLLGVLAARAARRRPEHLDTPDTPPRSQAQESNYENLSQMNPRSPPATMCSP

SEQ ID NO: 3 - DNA, 2458 bp, Homo sapiens
  misc_feature 1..2458: note = Homo sapiens myelin associated glycoprotein (MAG), transcript variant 1, mRNA
  source 1..2458: mol_type = genomic DNA
aggcggcccctggcacccagggggaggggaggggctggcaagtgggggcctagaccctggaaggcaggggactgcgagctgggctggcggagcagaggtgcagaagcaactgagtccaagttgtctggcggcttcaggtggacccagaagacgtccccaactcagggagattcagcgatcactcactcgctgtacagaatgatattcctcacggcactgcctctgttctggattatgatttcagcctcccgagggggtcactggggtgcctggatgccctcgtccatctcggccttcgaaggcacgtgcgtctccatcccctgccgctttgacttcccggatgagctgcggcccgctgtggtgcatggtgtctggtacttcaatagcccctaccccaagaactaccccccggtggtcttcaagtcgcgcacccaagtagtccacgagagcttccagggccgcagccgcctcctgggggacctgggcctgcgaaactgcaccctcctgctcagcaacgtcagccccgagctgggcgggaagtactacttccgtggggacctgggcggctacaaccagtacaccttctcagagcacagcgtcctggatatcgtcaacacccccaacatcgtggtgcccccagaggtggtggcaggcacggaggtggaggtcagctgcatggtgccggacaactgcccagagctgcgccctgagctgagctggctgggccacgaggggctgggggagcccgctgtgctgggccggctgcgggaggacgagggcacctgggtgcaggtgtcactgctgcacttcgtgcccacgagggaggccaacggccacaggctgggctgccaggcctccttccccaacaccaccctgcagttcgagggctacgccagcatggacgtcaagtaccccccggtgattgtggagatgaactcctcggtggaggccatcgagggctcccacgtgagcctgctctgtggggctgacagcaaccccccgccgctgctgacctggatgcgggacgggacagtcctccgggaggcggtggccgagagcctgctcctggagctggaggaggtgacccccgccgaagacggcgtctatgcctgcctggccgagaatgcctatggccaggacaaccgcaccgtggggctcagtgtcatgtatgcaccctggaagccaacagtgaacgggacaatggtggccgtagagggggagacggtctctatcttgtgctccacacagagcaacccggaccctattctcaccatcttcaaggagaagcagatcctgtccacggtcatctacgagagcgagctgcagctggagctgccggccgtgtcacccgaggatgatggagagtactggtgtgtggctgagaaccagtatggccagagggccaccgccttcaacctgtctgtggagttcgcccctgtgctcctcctggagtcccactgcgcggcagcccgagacacggtgcagtgcctgtgcgtggtgaagtccaacccggagccgtccgtggcctttgagctgccatcgcgcaatgtgaccgtgaacgagagcgagcgggagttcgtgtactcggagcgcagcggcctcgtgctcaccagcatcctcacgctgcgggggcaggcccaggccccgccccgcgtcatctgcaccgcgaggaacctctatggcgccaagagcctggagctgcccttccagggagcccatcgactgatgtgggccaagatcgggcctgtgggcgccgtggtcgcctttgccatcctgattgccatcgtctgctacattacccagacacgcaggaaaaagaacgtgacagagagccccagcttctcggcaggggacaaccctcccgtcctgttcagcagcgacttccgcatctctggggcaccagagaagtacgagagcgagaggcgcctgggatctgagaggaggctgctgggccttcggggtgagcccccagagctggacctgagctattctcactcggacctggggaaacggcccaccaaggacagctacacgctgacggaggagctagctgagtatgctgaaatccgggtcaagtgaaggagctgggggcagcctgcgtggctgacccccctcaggaccctcgctggcccccactggctgtgggctcccttcctcccaaaagtatcgggggctggggcaggaggggagtgaggcaggtgacagtgaggtcctgggggcctgacctccccctccttcccagctgcccctccctgccagcacccccacgccctcattacggctcctctctaacctcctttaccctcatctgtctggaggggagctctgtctgtccgtgttatttattgctacttcctgcctggtctcctgcccccacacctggccctggggcctgtacaaaagggacatgaaataaatgccccaaagccaaaaaaaaaaaaaaaaaaaaaaaaaaaaa

SEQ ID NO: 4 - protein, 626 aa, Homo sapiens
  REGION 1..626: note = misc_feature - myelin-associated glycoprotein isoform a precursor
MIFLTALPLFWIMISASRGGHWGAWMPSSISAFEGTCVSIPCRFDFPDELRPAVVHGVWYFNSPYPKNYPPVVFKSRTQVVHESFQGRSRLLGDLGLRNCTLLLSNVSPELGGKYYFRGDLGGYNQYTFSEHSVLDIVNTPNIVVPPEVVAGTEVEVSCMVPDNCPELRPELSWLGHEGLGEPAVLGRLREDEGTWVQVSLLHFVPTREANGHRLGCQASFPNTTLQFEGYASMDVKYPPVIVEMNSSVEAIEGSHVSLLCGADSNPPPLLTWMRDGTVLREAVAESLLLELEEVTPAEDGVYACLAENAYGQDNRTVGLSVMYAPWKPTVNGTMVAVEGETVSILCSTQSNPDPILTIFKEKQILSTVIYESELQLELPAVSPEDDGEYWCVAENQYGQRATAFNLSVEFAPVLLLESHCAAARDTVQCLCVVKSNPEPSVAFELPSRNVTVNESEREFVYSERSGLVLTSILTLRGQAQAPPRVICTARNLYGAKSLELPFQGAHRLMWAKIGPVGAVVAFAILIAIVCYITQTRRKKNVTESPSFSAGDNPPVLFSSDFRISGAPEKYESERRLGSERRLLGLRGEPPELDLSYSHSDLGKRPTKDSYTLTEELAEYAEIRVK

SEQ ID NO: 5 - DNA, 2626 bp, Homo sapiens
  misc_feature 1..2626: note = Homo sapiens leucine rich repeat containing 4C (LRRC4C), transcript variant 1, mRNA
  source 1..2626: mol_type = genomic DNA
agtttttggcttactttttggcggagtctcttggacacgtttttgctggtgctggaagatcagatacatggaacctttgaaaactgattatttttctccgatatgacttaaaaaaaaataaaaagaagaaaagaaaatagagtagtgcacggcaagctagaggattgtaaattttccttggtgaactttgaggatccataaagaaggagttactggaaaagcaagaataacttatgcggattaacaatatggaaacatcctgagactactttggaatcgccataaattaagtgggttccagttttgcaaacagagaaacgggtccatgaacaatttgctacaggtataaagaagtatctgcagaaatccagagcacttattaaacttctttgagttttctcaggaagatcaatacctgttggagaaattttactaagattggcaaacgcactgcctacttacagcatagagacccccagtggagagctagactgtttgaattccagaaggaccaacaccagataaattatgaatgttgaacaagatgaccttacatccacagcagataatgataggtcctaggtttaacagggccctatttgaccccctgcttgtggtgctgctggctcttcaacttcttgtggtggctggtctggtgcgggctcagacctgcccttctgtgtgctcctgcagcaaccagttcagcaaggtgatttgtgttcggaaaaacctgcgtgaggttccggatggcatctccaccaacacacggctgctgaacctccatgagaaccaaatccagatcatcaaagtgaacagcttcaagcacttgagacacttggaaatcctacagttgagtaggaaccatatcagaaccattgaaattggggctttcaatggtctggcgaacctcaacactctggaactctttgacaatcgtcttactaccatcccgaatggagcttttgtatacttgtctaaactgaaggagctctggttgcgaaacaaccccattgaaagcatcccttcttatgcttttaacagaattccttctttgcgccgactagacttaggggaattgaaaagactttcatacatctcagaaggtgcctttgaaggtctgtccaacttgaggtatttgaaccttgccatgtgcaaccttcgggaaatccctaacctcacaccgctcataaaactagatgagctggatctttctgggaatcatttatctgccatcaggcctggctctttccagggtttgatgcaccttcaaaaactgtggatgatacagtcccagattcaagtgattgaacggaatgcctttgacaaccttcagtcactagtggagatcaacctggcacacaataatctaacattactgcctcatgacctcttcactcccttgcatcatctagagcggatacatttacatcacaacccttggaactgtaactgtgacatactgtggctcagctggtggataaaagacatggccccctcgaacacagcttgttgtgcccggtgtaacactcctcccaatctaaaggggaggtacattggagagctcgaccagaattacttcacatgctatgctccggtgattgtggagccccctgcagacctcaatgtcactgaaggcatggcagctgagctgaaatgtcgggcctccacatccctgacatctgtatcttggattactccaaatggaacagtcatgacacatggggcgtacaaagtgcggatagctgtgctcagtgatggtacgttaaatttcacaaatgtaactgtgcaagatacaggcatgtacacatgtatggtgagtaattccgttgggaatactactgcttcagccaccctgaatgttactgcagcaaccactactcctttctcttacttttcaaccgtcacagtagagactatggaaccgtctcaggatgaggcacggaccacagataacaatgtgggtcccactccagtggtcgactgggagaccaccaatgtgaccacctctctcacaccacagagcacaaggtcgacagagaaaaccttcaccatcccagtgactgatataaacagtgggatcccaggaattgatgaggtcatgaagactaccaaaatcatcattgggtgttttgtggccatcacactcatggctgcagtgatgctggtcattttctacaagatgaggaagcagcaccatcggcaaaaccatcacgccccaacaaggactgttgaaattattaatgtggatgatgagattacgggagacacacccatggaaagccacctgcccatgcctgctatcgagcatgagcacctaaatcactataactcatacaaatctcccttcaaccacacaacaacagttaacacaataaattcaatacacagttcagtgcatgaaccgttattgatccgaatgaactctaaagacaatgtacaagagactcaaatctaaaacatttacagagttacaaaaaacaaacaatcaaaaaaaaagacagtttattaaaaatgacacaaatgactgggctaaatctactgtttcaaaaaagtgtctttacaaaaaaacaaaaaagaaaagaaatttatttattaaaaattctattgtgatctaaagcagacaaaa

SEQ ID NO: 6 - protein, 640 aa, Homo sapiens
  REGION 1..640: note = misc_feature - leucine-rich repeat-containing protein 4C precursor
MLNKMTLHPQQIMIGPRFNRALFDPLLVVLLALQLLVVAGLVRAQTCPSVCSCSNQFSKVICVRKNLREVPDGISTNTRLLNLHENQIQIIKVNSFKHLRHLEILQLSRNHIRTIEIGAFNGLANLNTLELFDNRLTTIPNGAFVYLSKLKELWLRNNPIESIPSYAFNRIPSLRRLDLGELKRLSYISEGAFEGLSNLRYLNLAMCNLREIPNLTPLIKLDELDLSGNHLSAIRPGSFQGLMHLQKLWMIQSQIQVIERNAFDNLQSLVEINLAHNNLTLLPHDLFTPLHHLERIHLHHNPWNCNCDILWLSWWIKDMAPSNTACCARCNTPPNLKGRYIGELDQNYFTCYAPVIVEPPADLNVTEGMAAELKCRASTSLTSVSWITPNGTVMTHGAYKVRIAVLSDGTLNFTNVTVQDTGMYTCMVSNSVGNTTASATLNVTAATTTPFSYFSTVTVETMEPSQDEARTTDNNVGPTPVVDWETTNVTTSLTPQSTRSTEKTFTIPVTDINSGIPGIDEVMKTTKIIIGCFVAITLMAAVMLVIFYKMRKQHHRQNHHAPTRTVEIINVDDEITGDTPMESHLPMPAIEHEHLNHYNSYKSPFNHTTTVNTINSIHSSVHEPLLIRMNSKDNVQETQI